European Patent Application EP 4 491 709 A1, published January 15, 2025. Title: A microorganism producing O-phosphoserine and a method for producing O-phosphoserine or L-methionine using the same. Applicant: CJ CheilJedang Corporation. The sequence listing filed with the application follows.

SEQUENCE LISTING (34 sequences)

SEQ ID NO: 1 - protein, 258 aa, Corynebacterium glutamicum
MSERQLEKSIEHAVELAREARNIEVFTGAGMSADSGLETYRDDKTGLWSNVDPQAMASIDAWRKDPEPMWAWYRWRAGVAARAEPNAGHQAISYWEGSDTVEHVHITTQNIDNLHERAGSSDVTHLHGSLFEYRCSDCATPWEDDKNYPQEPIARLAPPQCEKCGGLIRPGVVWFGENLPVEEWDIAEQRIAEADLMIIVGTSGIVHPAAALPQLAQQRGVPIVEISPTRTELSRIADFTWMSTAAQALPALMRGLSA

SEQ ID NO: 2 - protein, 195 aa, Corynebacterium glutamicum
MVELEQHGFLSGVVTQNVDGLHAEAGTKNLVALHGDLAHVMCLNCGFGEDRHLFDERLEAANPGYVASIRLEPGAVNPDGDVFLDEEQVRRFTMIGCLRCGSLMLKPDVVYFGEPVPAARKKDLKKLLDASSSLLIAGSSLAVMSGYRIVIEAQRQGKQVSVINGGPGRADSRVDILWRTRVAPAFDDILDALDL

SEQ ID NO: 3 - DNA, 36 bp, synthetic construct
  misc_feature 1..36: note = 0616 _del up F
  source 1..36: mol_type = other DNA
tcgagctcggtacccagcataattccatactcccac

SEQ ID NO: 4 - DNA, 42 bp, synthetic construct
  misc_feature 1..42: note = 0616 _del up R
  source 1..42: mol_type = other DNA
ggtagcgcttgggctgcagtactctcgacggcgtgctcaatt

SEQ ID NO: 5 - DNA, 42 bp, synthetic construct
  misc_feature 1..42: note = 0616 _del down F
  source 1..42: mol_type = other DNA
aattgagcacgccgtcgagagtactgcagcccaagcgctacc

SEQ ID NO: 6 - DNA, 34 bp, synthetic construct
  misc_feature 1..34: note = 0616 _del down R
  source 1..34: mol_type = other DNA
ctctagaggatccccctacgacgctactgcgcag

SEQ ID NO: 7 - DNA, 5803 bp, synthetic construct
  misc_feature 1..5803: note = pDCM2
  source 1..5803: mol_type = other DNA
gttcgcttgctgtccataaaaccgcccagtctagctatcgccatgtaagcccactgcaagctacctgctttctctttgcgcttgcgttttcccttgtccagatagcccagtagctgacattcatccggggtcagcaccgtttctgcggactggctttctacgtgttccgcttcctttagcagcccttgcgccctgagtgcttgcggcagcgtgaagctagcttttatcgccattcgccattcaggctgcgcaactgttgggaagggcgatcggtgcgggcctcttcgctattacgccagctggcgaaagggggatgtgctgcaaggcgattaagttgggtaacgccagggttttcccagtcacgacgttgtaaaacgacggccagtgaattcgagctcggtacccggggatcctctagagtcgacctgcaggcatgcaagcttggcgtaatcatggtcatagctgtttcctgtgtgaaattgttatccgctcacaattccacacaacatacgagccggaagcataaagtgtaaagcctggggtgcctaatgagtgagctaactcacattaattgcgttgcgctcactgcccgctttccagtcgggaaacctgtcgtgccagctgcattaatgaatcggccaacgcgcggggagaggcggtttgcgtattgggcgctcttccgcttcctcgctcactgactcgctgcgctcggtcgttcggctgcggcgagcggtatcagctcactcaaaggcggtaatacggttatccacagaatcaggggataacgcaggaaagaacatgtgagcaaaaggccagcaaaaggccaggaaccgtaaaaaggccgcgttgctggcgtttttccataggctccgcccccctgacgagcatcacaaaaatcgacgctcaagtcagaggtggcgaaacccgacaggactataaagataccaggcgtttccccctggaagctccctcgtgcgctctcctgttccgaccctgccgcttaccggatacctgtccgcctttctcccttcgggaagcgtggcgctttctcaatgctcacgctgtaggtatctcagttcggtgtaggtcgttcgctccaagctgggctgtgtgcacgaaccccccgttcagcccgaccgctgcgccttatccggtaactatcgtcttgagtccaacccggtaagacacgacttatcgccactggcagcagccactggtaacaggattagcagagcgaggtatgtaggcggtgctacagagttcttgaagtggtggcctaactacggctacactagaaggacagtatttggtatctgcgctctgctgaagccagttaccttcggaaaaagagttggtagctcttgatccggcaaacaaaccaccgctggtagcggtggtttttttgtttgcaagcagcagattacgcgcagaaaaaaaggatctcaagaagatcctttgatcttttctacggggtctgacgctcagtggaacgaaaactcacgttaagggattttggtcatgagattatcaaaaaggatcttcacctagatccttttggggtgggcgaagaactccagcatgagatccccgcgctggaggatcatccagccctgatagaaacagaagccactggagcacctcaaaaacaccatcatacactaaatcagtaagttggcagcatcacccgacgcactttgcgccgaataaatacctgtgacggaagatcacttcgcagaataaataaatcctggtgtccctgttgataccgggaagccctgggccaacttttggcgaaaatgagacgttgatcggcacgtaagaggttccaactttcaccataatgaaataagatcactaccgggcgtattttttgagttatcgagattttcaggagctgatagaaacagaagccactggagcacctcaaaaacaccatcatacactaaatcagtaagttggcagcatcacccgacgcactttgcgccgaataaatacctgtgacggaagatcacttcgcagaataaataaatcctggtgtccctgttgataccgggaagccctgggccaacttttggcgaaaatgagacgttgatcggcacgtaagaggttccaactttcaccataatgaaataagatcactaccgggcgtattttttgagttatcgagattttcaggagctctttggcatcgtctctcgcctgtcccctcagttcagtaatttcctgcatttgcctgtttccagtcggtagatattccacaaaacagcagggaagcagcgcttttccgctgcataaccctgcttcggggtcattatagcgattttttcggtatatccatcctttttcgcacgatatacaggattttgccaaagggttcgtgtagactttccttggtgtatccaacggcgtcagccgggcaggataggtgaagtaggcccacccgcgagcgggtgttccttcttcactgtcccttattcgcacctggcggtgctcaacgggaatcctgctctgcgaggctggccggctaccgccggcgtaacagatgagggcaagcggatggctgatgaaaccaagccaaccaggaagggcagcccacctatcaaggtgtactgccttccagacgaacgaagagcgattgaggaaaaggcggcggcggccggcatgagcctgtcggcctacctgctggccgtcggccagggctacaaaatcacgggcgtcgtggactatgagcacgtccgcgagggcgtcccggaaaacgattccgaagcccaacctttcatagaaggcggcggtggaatcgaaatctcgtgatggcaggttgggcgtcgcttggtcggtcatttcgaaaaaggttaggaatacggttagccatttgcctgcttttatatagttcantatgggattcacctttatgttgataagaaataaaagaaaatgccaataggatatcggcattttcttttgcgtttttatttgttaactgttaattgtccttgttcaaggatgctgtctttgacaacagatgttttcttgcctttgatgttcagcaggaagctcggcgcaaacgttgattgtttgtctgcgtagaatcctctgtttgtcatatagcttgtaatcacgacattgtttcctttcgcttgaggtacagcgaagtgtgagtaagtaaaggttacatcgttaggcggatcaagatccatttttaacacaaggccagttttgttcagcggcttgtatgggccagttaaagaattagaaacataaccaagcatgtaaatatcgttagacgtaatgccgtcaatcgtcatttttgatccgcgggagtcagtgaacaggtaccatttgccgttcattttaaagacgttcgcgcgttcaatttcatctgttactgtgttagatgcaatcagcggtttcatcacttttttcagtgtgtaatcatcgtttagctcaatcataccgagagcgccgtttgctaactcagccgtgcgttttttatcgctttgcagaagtttttgactttcttgacggaagaatgatgtgcttttgccatagtatgctttgttaaataaagattcttcgccttggtagccatcttcagttccagtgtttgcttcaaatactaagtatttgtggcctttatcttctacgtagtgaggatctctcagcgtatggttgtcgcctgagctgtagttgccttcatcgatgaactgctgtacattttgatacgtttttccgtcaccgtcaaagattgatttataatcctctacaccgttgatgttcaaagagctgtctgatgctgatacgttaacttgtgcagttgtcagtgtttgtttgccgtaatgtttaccggagaaatcagtgtagaataaacggatttttccgtcagatgtaaatgtggctgaacctgaccattcttgtgtttggtcttttaggatagaatcatttgcatcgaatttgtcgctgtctttaaagacgcggccagcgtttttccagctgtcaatagaagtttcgccgactttttgatagaacatgtaaatcgatgtgtcatccgcatttttaggatctccggctaatgcaaagacgatgtggtagccgtgatagtttgcgacagtgccgtcagcgttttgtaatggccagctgtcccaaacgtccaggccttttgcagaagagatatttttaattgtggacgaatcaaattcagaaacttgatatttttcatttttttgctgttcagggatttgcagcatatcatggcgtgtaatatgggaaatgccgtatgtttccttatatggcttttggttcgtttctttcgcaaacgcttgagttgcgcctcctgccagcagtgcggtagtaaaggttaatactgttgcttgttttgcaaactttttgatgttcatcgttcatgtctccttttttatgtactgtgttagcggtctgcttcttccagccctcctgtttgaagatggcaagttagttacgcacaataaaaaaagacctaaaatatgtaaggggtgacgccaaagtatacactttgccctttacacattttaggtcttgcctgctttatcagtaacaaacccgcgcgatttacttttcgacctcattctattagactctcgtttggattgcaactggtctattttcctcttttgtttgatagaaaatcataaaaggatttgcagactacgggcctaaagaactaaaaaatctatctgtttcttttcattctctgtattttttatagtttctgttgcatgggcataaagttgcctttttaatcacaattcagaaaatatcataatatctcatttcactaaataatagtgaacggcaggtatatgtgatgggttaaaaaggatcaccccagagtcccgctcagaagaactcgtcaagaaggcgatagaaggcgatgcgctgcgaatcgggagcggcgataccgtaaagcacgaggaagcggtcagcccattcgccgccaagctcttcagcaatatcacgggtagccaacgctatgtcctgatagcggtccgccacacccagccggccacagtcgatgaatccagaaaagcggccattttccaccatgatattcggcaagcaggcatcgccatgggtcacgacgagatcctcgccgtcgggcatccgcgccttgagcctggcgaacagttcggctggcgcgagcccctgatgctcttcgtccagatcatcctgatcgacaagaccggcttccatccgagtacgtgctcgctcgatgcgatgtttcgcttggtggtcgaatgggcaggtagccggatcaagcgtatgcagccgccgcattgcatcagccatgatggatactttctcggcaggagcaaggtgagatgacaggagatcctgccccggcacttcgcccaatagcagccagtcccttcccgcttcagtgacaacgtcgagacagctgcgcaaggaacgcccgtcgtggccagccacgatagccgcgctgcctcgtcttggagttcattcagggcaccggacaggtcggtcttgacaaaaagaaccgggcgcccctgcgctgacagccggaacacggcggcatcagagcagccgattgtctgttgtgcccagtcatagccgaatagcctctccacccaagcggccggagaacctgcgtgcaatccatcttgttcaatcatgcgaaacgatcctcatcctgtctcttgatcagatcttgatcccctgcgccatcagatccttggcggcaagaaagccatccagtttactttgcagggcttcccaaccttaccagagggcgccccagctggcaattccg

SEQ ID NO: 8 - DNA, 18 bp, synthetic construct
  misc_feature 1..18: note = 0616 _del F
  source 1..18: mol_type = other DNA
ggcttccaactgtaatgg

SEQ ID NO: 9 - DNA, 18 bp, synthetic construct
  misc_feature 1..18: note = 0616 _del R
  source 1..18: mol_type = other DNA
tagaacacccagctaaca

SEQ ID NO: 10 - protein, 418 aa, synthetic construct
  REGION 1..418: note = YjeH F351L
MSGLKQELGLAQGIGLLSTSLLGTGVFAVPALAALVAGNNSLWAWPVLIILVFPIAIVFAILGRHYPSAGGVAHFVGMAFGSRLERVTGWLFLSVIPVGLPAALQIAAGFGQAMFGWHSWQLLLAELGTLALVWYIGTRGASSSANLQTVIAGLIVALIVAIWWAGDIKPANIPFPAPGNIELTGLFAALSVMFWCFVGLEAFAHLASEFKNPERDFPRALMIGLLLAGLVYWGCTVVVLHFDAYGEKMAAAASLPKIVVQLFGVGALWIACVIGYLACFASLNIYIQSFARLVWSQAQHNPDHYLARLSSRHIPNNALNAVLGCCVVSTLVIHALEINLDALIIYANGILIMIYLLCMLAGCKLLQGRYRLLAVVGGLLCVLLLAMVGWKSLYALIMLAGLWLLLPKRKTPENGITT

SEQ ID NO: 11 - DNA, 1161 bp, unidentified
  misc_feature 1..1161: note = Corynebacterium glutamicum metB
  source 1..1161: mol_type = genomic DNA
ttgtcttttgacccaaacacccagggtttctccactgcatcgattcacgctgggtatgagccagacgactactacggttcgattaacaccccaatctatgcctccaccaccttcgcgcagaacgctccaaacgaactgcgcaaaggctacgagtacacccgtgtgggcaaccccaccatcgtggcattagagcagaccgtcgcagcactcgaaggcgcaaagtatggccgcgcattctcctccggcatggctgcaaccgacatcctgttccgcatcatcctcaagccgggcgatcacatcgtcctcggcaacgatgcttacggcggaacctaccgcctgatcgacaccgtattcaccgcatggggcgtcgaatacaccgttgttgatacctccgtcgtggaagaggtcaaggcagcgatcaaggacaacaccaagctgatctgggtggaaaccccaaccaacccagcacttggcatcaccgacatcgaagcagtagcaaagctcaccgaaggcaccaacgccaagctggttgttgacaacaccttcgcatccccatacctgcagcagccactaaaactcggcgcacacgcagtcctgcactccaccaccaagtacatcggaggacactccgacgttgttggcggccttgtggttaccaacgaccaggaaatggacgaagaactgctgttcatgcagggcggcatcggaccgatcccatcagttttcgatgcatacctgaccgcccgtggcctcaagacccttgcagtgcgcatggatcgccactgcgacaacgcagaaaagatcgcggaattcctggactcccgcccagaggtctccaccgtgctctacccaggtctgaagaaccacccaggccacgaagtcgcagcgaagcagatgaagcgcttcggcggcatgatctccgtccgtttcgcaggcggcgaagaagcagctaagaagttctgtacctccaccaaactgatctgtctggccgagtccctcggtggcgtggaatccctcctggagcacccagcaaccatgacccaccagtcagctgccggctctcagctcgaggttccccgcgacctcgtgcgcatctccattggtattgaagacattgaagacctgctcgcagatgtcgagcaggccctcaataacctttag

SEQ ID NO: 12 - DNA, 18 bp, synthetic construct
  misc_feature 1..18: note = metB_N_del F
  source 1..18: mol_type = other DNA
ggcttcggagttggagcg

SEQ ID NO: 13 - DNA, 40 bp, synthetic construct
  misc_feature 1..40: note = metB_N_del R
  source 1..40: mol_type = other DNA
gccaaatagtttcccgggggtagatcaactcctgtaatca

SEQ ID NO: 14 - DNA, 40 bp, synthetic construct
  misc_feature 1..40: note = metB_C_del F
  source 1..40: mol_type = other DNA
caggagttgatctacccccgggaaactatttggcggcaag

SEQ ID NO: 15 - DNA, 19 bp, synthetic construct
  misc_feature 1..19: note = metB_C_del R
  source 1..19: mol_type = other DNA
tcgcgtctgggtgcgcatc

SEQ ID NO: 16 - DNA, 1314 bp, unidentified
  misc_feature 1..1314: note = Corynebacterium glutamicum metY
  source 1..1314: mol_type = genomic DNA
atgccaaagtacgacaattccaatgctgaccagtggggctttgaaacccgctccattcacgcaggccagtcagtagacgcacagaccagcgcacgaaaccttccgatctaccaatccaccgctttcgtgttcgactccgctgagcacgccaagcagcgtttcgcacttgaggatctaggccctgtttactcccgcctcaccaacccaaccgttgaggctttggaaaaccgcatcgcttccctcgaaggtggcgtccacgctgtagcgttctcctccggacaggccgcaaccaccaacgccattttgaacctggcaggagcgggcgaccacatcgtcacctccccacgcctctacggtggcaccgagactctattccttatcactcttaaccgcctgggtatcgatgtttccttcgtggaaaaccccgacgaccctgagtcctggcaggcagccgttcagccaaacaccaaagcattcttcggcgagactttcgccaacccacaggcagacgtcctggatattcctgcggtggctgaagttgcgcaccgcaacagcgttccactgatcatcgacaacaccatcgctaccgcagcgctcgtgcgcccgctcgagctcggcgcagacgttgtcgtcgcttccctcaccaagttctacaccggcaacggctccggactgggcggcgtgcttatcgacggcggaaagttcgattggactgtcgaaaaggatggaaagccagtattcccctacttcgtcactccagatgctgcttaccacggattgaagtacgcagaccttggtgcaccagccttcggcctcaaggttcgcgttggccttctacgcgacaccggctccaccctctccgcattcaacgcatgggctgcagtccagggcatcgacaccctttccctgcgcctggagcgccacaacgaaaacgccatcaaggttgcagaattcctcaacaaccacgagaaggtggaaaaggttaacttcgcaggcctgaaggattccccttggtacgcaaccaaggaaaagcttggcctgaagtacaccggctccgttctcaccttcgagatcaagggcggcaaggatgaggcttgggcatttatcgacgccctgaagctacactccaaccttgcaaacatcggcgatgttcgctccctcgttgttcacccagcaaccaccacccattcacagtccgacgaagctggcctggcacgcgcgggcgttacccagtccaccgtccgcctgtccgttggcatcgagaccattgatgatatcatcgctgacctcgaaggcggctttgctgcaatctag

SEQ ID NO: 17 - DNA, 18 bp, synthetic construct
  misc_feature 1..18: note = metY_N_del F
  source 1..18: mol_type = other DNA
ccaaagacaaggagacca

SEQ ID NO: 18 - DNA, 40 bp, synthetic construct
  misc_feature 1..40: note = metY_N_del R
  source 1..40: mol_type = other DNA
agtctatttaaagcccgggttggaggtccttaagagtttt

SEQ ID NO: 19 - DNA, 40 bp, synthetic construct
  misc_feature 1..40: note = metY_C_del F
  source 1..40: mol_type = other DNA
taaggacctccaacccgggctttaaatagactcaccccag

SEQ ID NO: 20 - DNA, 18 bp, synthetic construct
  misc_feature 1..18: note = metY_C_del R
  source 1..18: mol_type = other DNA
atgccgagtgcgtcgagg

SEQ ID NO: 21 - DNA, 1266 bp, unidentified
  misc_feature 1..1266: note = Corynebacterium glutamicum lysC
  source 1..1266: mol_type = genomic DNA
gtggccctggtcgtacagaaatatggcggttcctcgcttgagagtgcggaacgcattagaaacgtcgctgaacggatcgttgccaccaagaaggctggaaatgatgtcgtggttgtctgctccgcaatgggagacaccacggatgaacttctagaacttgcagcggcagtgaatcccgttccgccagctcgtgaaatggatatgctcctgactgctggtgagcgtatttctaacgctctcgtcgccatggctattgagtcccttggcgcagaagcccaatctttcacgggctctcaggctggtgtgctcaccaccgagcgccacggaaacgcacgcattgttgatgtcactccaggtcgtgtgcgtgaagcactcgatgagggcaagatctgcattgttgctggtttccagggtgttaataaagaaacccgcgatgtcaccacgttgggtcgtggtggttctgacaccactgcagttgcgttggcagctgctttgaacgctgatgtgtgtgagatttactcggacgttgacggtgtgtataccgctgacccgcgcatcgttcctaatgcacagaagctggaaaagctcagcttcgaagaaatgctggaacttgctgctgttggctccaagattttggtgctgcgcagtgttgaatacgctcgtgcattcaatgtgccacttcgcgtacgctcgtcttatagtaatgatcccggcactttgattgccggctctatggaggatattcctgtggaagaagcagtccttaccggtgtcgcaaccgacaagtccgaagccaaagtaaccgttctgggtatttccgataagccaggcgaggctgcgaaggttttccgtgcgttggctgatgcagaaatcaacattgacatggttctgcagaacgtctcttctgtagaagacggcaccaccgacatcaccttcacctgccctcgttccgacggccgccgcgcgatggagatcttgaagaagcttcaggttcagggcaactggaccaatgtgctttacgacgaccaggtcggcaaagtctccctcgtgggtgctggcatgaagtctcacccaggtgttaccgcagagttcatggaagctctgcgcgatgtcaacgtgaacatcgaattgatttccacctctgagattcgtatttccgtgctgatccgtgaagatgatctggatgctgctgcacgtgcattgcatgagcagttccagctgggcggcgaagacgaagccgtcgtttatgcaggcaccggacgctaa

SEQ ID NO: 22 - DNA, 19 bp, synthetic construct
  misc_feature 1..19: note = lysC_L377K_5 F
  source 1..19: mol_type = other DNA
cagaagctggaaaagctca

SEQ ID NO: 23 - DNA, 40 bp, synthetic construct
  misc_feature 1..40: note = lysC_L377K_5 R
  source 1..40: mol_type = other DNA
atctcagaggtggaaatcttttcgatgttcacgttgacat

SEQ ID NO: 24 - DNA, 40 bp, synthetic construct
  misc_feature 1..40: note = lysC_L377K_3 F
  source 1..40: mol_type = other DNA
tgtcaacgtgaacatcgaaaagatttccacctctgagatt

SEQ ID NO: 25 - DNA, 19 bp, synthetic construct
  misc_feature 1..19: note = lysC_L377K_3 R
  source 1..19: mol_type = other DNA
tccttgtcggaagggttca

SEQ ID NO: 26 - DNA, 1134 bp, unidentified
  misc_feature 1..1134: note = Corynebacterium glutamicum metX
  source 1..1134: mol_type = genomic DNA
atgcccaccctcgcgccttcaggtcaacttgaaatccaagcgatcggtgatgtctccaccgaagccggagcaatcattacaaacgctgaaatcgcctatcaccgctggggtgaataccgcgtagataaagaaggacgcagcaatgtcgttctcatcgaacacgccctcactggagattccaacgcagccgattggtgggctgacttgctcggtcccggcaaagccatcaacactgatatttactgcgtgatctgtaccaacgtcatcggtggttgcaacggttccaccggacctggctccatgcatccagatggaaatttctggggtaatcgcttccccgccacgtccattcgtgatcaggtaaacgccgaaaaacaattcctcgacgcactcggcatcaccacggtcgccgcagtacttggtggttccatgggtggtgcccgcaccctagagtgggccgcaatgtacccagaaactgttggcgcagctgctgttcttgcagtttctgcacgcgccagcgcctggcaaatcggcattcaatccgcccaaattaaggcgattgaaaacgaccaccactggcacgaaggcaactactacgaatccggctgcaacccagccaccggactcggcgccgcccgacgcatcgcccacctcacctaccgtggcgaactagaaatcgacgaacgcttcggcaccaaagcccaaaagaacgaaaacccactcggtccctaccgcaagcccgaccagcgcttcgccgtggaatcctacttggactaccaagcagacaagctagtacagcgtttcgacgccggctcctacgtcttgctcaccgacgccctcaaccgccacgacattggtcgcgaccgcggaggcctcaacaaggcactcgaatccatcaaagttccagtccttgtcgcaggcgtagataccgatattttgtacccctaccaccagcaagaacacctctccagaaacctgggaaatctactggcaatggcaaaaatcgtatcccctgtcggccacgatgctttcctcaccgaaagccgccaaatggatcgcatcgtgaggaacttcttcagcctcatctccccagacgaagacaacccttcgacctacatcgagttctacatctaa

SEQ ID NO: 27 - DNA, 28 bp, synthetic construct
  misc_feature 1..28: note = metX F
  source 1..28: mol_type = other DNA
ggatcccctcgttgttcacccagcaacc

SEQ ID NO: 28 - DNA, 30 bp, synthetic construct
  misc_feature 1..30: note = metX R
  source 1..30: mol_type = other DNA
ggatcccaaagtcacaactacttatgttag

SEQ ID NO: 29 - DNA, 777 bp, Corynebacterium glutamicum
  source 1..777: mol_type = genomic DNA
atgagcgaacgtcagctggaaaagtcaattgagcacgccgtcgagttagcccgcgaagcccgaaacatcgaagtttttaccggagccggaatgagcgccgactccgggttggaaacgtatcgtgatgataaaaccgggctgtggagcaacgtagatccacaagcgatggcaagtatcgatgcatggcgcaaagatccagagccaatgtgggcgtggtatcgctggcgcgccggggtggcagctagggcagaacccaacgcggggcatcaagctatttcctactgggaggggagtgacaccgtcgaacacgttcacatcaccacccagaacattgacaacctgcacgagcgagctggctctagcgatgtgacacatcttcatggcagcttgtttgaatacaggtgctctgattgtgcgactccatgggaagacgataaaaactatccgcaagaacccattgcacgccttgctcctccacaatgtgaaaagtgcggagggctgattagaccaggtgtggtgtggtttggtgagaacctgcccgtagaagagtgggatattgcagagcaacgcatcgcagaagccgatctcatgatcattgtgggtacctccgggattgttcatcctgcagcagcactcccgcaattagcccaacaacgcggcgttcccatcgtggagatctccccaacgcgcaccgaacttagccggatcgcagacttcacctggatgtccaccgcagcccaagcgctaccagcgttgatgcgaggtttgagcgcctaa

SEQ ID NO: 30 - DNA, 588 bp, Corynebacterium glutamicum
  source 1..588: mol_type = genomic DNA
atggttgagctggagcagcatggttttttaagtggtgtggtcacccaaaatgtcgatggtttacacgcggaagcaggcacgaaaaacctggtcgcgctgcatggtgatctcgcccatgtgatgtgtttgaactgcggtttcggggaggatcgacacctctttgatgaacgtctcgaagccgccaaccccggctacgtcgcttccattcgcctggaaccgggcgcagtcaaccccgacggcgacgtcttcctcgacgaagaacaagtacgccgcttcaccatgatcggctgcttgcgctgcggctcgctcatgctcaaaccagacgtggtttacttcggcgaacccgtgcccgccgcgcgcaaaaaagatttaaaaaagcttctcgacgcctcctccagcctcttaatcgccggctcctccctagccgtcatgagtggataccggatcgtcatcgaagcgcaacgtcaaggaaaacaagtgtctgtcatcaacggcggcccaggtcgggcggattcccgcgtggacattttgtggcgcacccgcgttgcaccggcctttgatgacattttggacgcgctggacctttag

SEQ ID NO: 31 - DNA, 42 bp, synthetic construct
  misc_feature 1..42: note = 0078 _del up F
  source 1..42: mol_type = other DNA
gtgaattcgagctcggtacccttagccttgtccgagaacctc

SEQ ID NO: 32 - DNA, 42 bp, synthetic construct
  misc_feature 1..42: note = 0078 _del up R
  source 1..42: mol_type = other DNA
aagccaccaaaagtcccgggtcccctatcctaagccacatct

SEQ ID NO: 33 - DNA, 42 bp, synthetic construct
  misc_feature 1..42: note = 0078 _del down F
  source 1..42: mol_type = other DNA
gcttaggataggggacccgggacttttggtggcttaagttcg

SEQ ID NO: 34 - DNA, 42 bp, synthetic construct
  misc_feature 1..42: note = 0078 _del down R
  source 1..42: mol_type = other DNA
ggtcgactctagaggatcccctaccaactgcgggagttacta